European Patent Specification EP 3 699 592 B1, published April 29, 2026. Title: NON-REPLICATIVE TRANSDUCTION PARTICLES AND TRANSDUCTION PARTICLE-BASED REPORTER SYSTEMS. Applicant: GENEWEAVE BIOSCIENCES, INC. Application PCT/US2014/026536. The sequence listing filed with the application follows.

SEQUENCE LISTING (22 sequences)

SEQ ID NO: 1 - DNA, 177 bp, Enterobacteria phage P1
ccactaaaaagcatgatcattgatcactctaatgatcaacatgcaggtgatcacattgcggctgaaatagcggaaaaacaaagagttaatgccgttgtcagtgccgcagtcgagaatgcgaagcgccaaaataagcgcataaatgatcgttcagatgatcatgacgtgatcacccgc

SEQ ID NO: 2 - DNA, 177 bp, Artificial Sequence
  Description of Artificial Sequence: Synthetic polynucleotide
ccactaaaaagcatgataatagaccactctaacgaccaacatgcaggggagcacattgcggctgaaatagcggaaaagcagagggtgaatgccgttgtcagtgccgcagtcgagaatgcgaagcgccaaaataagcgcataaacgaccgttcagacgaccatgacgttattacccgc

SEQ ID NO: 3 - DNA, 1727 bp, Artificial Sequence
  Description of Artificial Sequence: Synthetic polynucleotide
cactatagggcgaattggcggaaggccgtcaaggccgcatttgggcccggcgcgccggatccgctagctctagactggcaggtttctgagcagatcgtccaacccgatctggatcgggtcagaaaaatttgctctaataaatttcgttttctaagtgcaaagaatcaccatttcgagctggtgattgaaggttgatgcaaatttggagaaaaaatgcaacaaacattcaatgcggatatgaatatatcaaaccttcatcaaaatgtcgatccttcaaccactctgcccgttatttgtggtgttgaaattacgaccgaccgcgctggccgttacaaccttaatgctctacacagagcgagcggactcggtgcccataaagcgccagctcaatggctaagaacgctgtcagctaaacagctcatcgaagagcttgaaaaagaaactatgcagaattgcatagtttcgttcacaagcaatggaagcaggatttctttcacgactcgtataaccggcaaaggtcagcagtggctgatgaagcgattgcttgatgctggtgtgctggtacctgtcgcggcaacgcgctaacagacgtagtaagaaccaccagcattgtaatgctggctaaagtcactttcctgagctgtataacgatgagcgattttactttttctggctatgaattggcctgctttgtaacacactccggtctatcccgtagcgccgggcatatcctgtcgcaatgtgcaaatctcgcggcaacaaccagtgaatacttcattcacaagcctcaccgcctgatcgcggcagaaactggttatagccaatcaaccgtcgttcgtgcattccgtgaagctgtaaacaaaggaattctgtctgtagagattgttatcggcgatcaccgtgaacgtcgcgctaacctgtaccggtttacaccatcctttttggccttcgcacaacaagccaaaaatgcgctgatagaaagcaaattaaagatctcttcagcggcaaccaaggttaaagctgttctcgctaagacattggctttatttaattttttatccacacccccatgtcaaaatgataccccctccccctgtcaggatgacgtggcaataaagaataagaagtcacaagttaaaaaaacaaaaagatcagtttccggcggtgccggaacaaccagcctcaaaaaattgacttcatggatcgctaaggcaaaagcaaaggctgacaatctgcggttatccaaaaaacgcactcaaaaacatgagttcaagcagaaagtagaggcggctgcgcggaaatatgcttacctgaagaacaagcgttcgcctgatattggcgggatatcaaacttcgataacctaccgcattgcatgacggtaaacgaagctcttaatgcggttttagccaaaaataaagataacgaacaatggggtataccggcaggattcagagggtaatgaattgctctaattataaccatgcatactttcaacacctctagtttgccatgaggcaaactcataggtgtcctggtaagaggacactgttgccaaaactggacgccccattattgcaattaataaacaactaacggacaattctacctaacaataagtggcttaaaaaaacccgccccggcgggtttttttatctagagctagcggatccggcgcgccgggcccttctgggcctcatgggccttccgctcactgcccgctttccag

SEQ ID NO: 4 - DNA, 131 bp, Artificial Sequence
  Description of Artificial Sequence: Synthetic polynucleotide
cgtcaggtggcacttttcgggaaatgtgcgcggaacccctatttgtttattttctaaatacattcaaatatgtatccgctcatgagacaataaccctgataaatgcttcaataatattgaaaaggaagagt

SEQ ID NO: 5 - DNA, 4681 bp, Artificial Sequence
  Description of Artificial Sequence: Synthetic polynucleotide
  modified_base (301)..(301): a, c, t, g, unknown or other
  modified_base (4056)..(4056): a, c, t, g, unknown or other
tttgcggaaagagttagtaagttaacagaagacgagccaaacctaaatggtttagcaggaaacttagataaaaaaatgaatccagaattatattcagaacaggaacagcaacaagagcaacaaaagaatcaaaaacgagatagaggtatgcacttatagaacatgcatttatgccgagaaaacttattggttggaatgggctatgtgttagctaacttgttagcgagttggttggacttgaattgggattaatcccaagaaagtaccggctcaacaacccataaagccctgtaggttccgnccaataaggaaattggaataaagcaataaaaggagttgaagaaatgaaattcagagaagcctttgagaattttataacaagtaagtatgtacttggtgttttagtagtcttaactgtttaccagataatacaaatgcttaaataaaaaaagacttgatctgattagaccaaatcttttgatagtgttatattaataacaaaataaaaaggagtcgctcacgccctaccaaagtttgtgaacgacatcattcaaagaaaaaaacactgagttgtttttataatcttgtatatttagatattaaacgatatttaaatatacatcaagatatatatttgggtgagcgattacttaaacgaaattgagattaaggagtcgattttttatgtataaaaacaatcatgcaaatcattcaaatcatttggaaaatcacgatttagacaatttttctaaaaccggctactctaatagccggttggacgcacatactgtgtgcatatctgatccaaaattaagttttgatgcaatgacgatcgttggaaatctcaaccgagacaacgctcaggccctttctaaatttatgagtgtagagccccaaataagactttgggatattcttcaaacaaagtttaaagctaaagcacttcaagaaaaagtttatattgaatatgacaaagtgaaagcagatagttgggatagacgtaatatgcgtattgaatttaatccaaacaaacttacacgagatgaaatgatttggttaaaacaaaatataataagctacatggaagatgacggttttacaagattagatttagcctttgattttgaagatgatttgagtgactactatgcaatgtctgataaagcagttaagaaaactattttttatggtcgtaatggtaagccagaaacaaaatattttggcgtgagagatagtaatagatttattagaatttataataaaaagcaagaacgtaaagataatgcagatgctgaagttatgtctgaacatttatggcgtgtagaaatcgaacttaaaagagatatggtggattactggaatgattgctttagtgatttacatatcttgcaaccagattggaaaactatccaacgcactgcggatagagcaatagtttttatgttattgagtgatgaagaagaatggggaaagcttcacagaaattctagaacaaaatataagaatttgataaaagaaatttcgccagtcgatttaacggacttaatgaaatcgactttaaaagcgaacgaaaaacaattgcaaaaacaaatcgatttttggcaacatgaatttaaattttggaaatagtgtacatattaatattactgaacaaaaatgatatatttaaactattctaatttaggaggatttttttatgaagtgtctatttaaaaatttggggaatttatatgaggtgaaagaataatttacccctataaactttagccacctcaagtaaagaggtaaaattgtttagtttatataaaaaatttaaaggtttgttttatagcgttttattttggctttgtattctttcattttttagtgtattaaatgaaatggttttaaatgtttctttacctgatattgcaaatcattttaatactactcctggaattacaaactgggtaaacactgcatatatgttaactttttcgataggaacagcagtatatggaaaattatctgattatataaatataaaaaaattgttaattattggtattagtttgagctgtcttggttcattgattgcttttattgggcccacctaggcaaatatgctcttacgtgctattatttaagtgactatttaaaaggagttaataaatatgcggcaaggtattcttaaataaactgtcaatttgatagcgggaacaaataattagatgtccttttttaggagggcttagttttttgtacccagtttaagaatacctttatcatgtgattctaaagtatccagagaatatctgtatgctttgtatacctatggttatgcataaaaatcccagtgataaaagtatttatcactgggatttttatgcccttttgggtttttgaatggaggaaaatcacatgaaaattattaatattggagttttagctcatgttgatgcaggaaaaactaccttaacagaaagcttattatataacagtggagcgattacagaattaggaagcgtggacaaaggtacaacgaggacggataatacgcttttagaacgtcagagaggaattacaattcagacaggaataacctcttttcagtgggaaaatacgaaggtgaacatcatagacacgccaggacatatggatttcttagcagaagtatatcgttcattatcagttttagatggggcaattctactgatttctgcaaaagatggcgtacaagcacaaactcgtatattatttcatgcacttaggaaaatggggattcccacaatcttttttatcaataagattgaccaaaatggaattgatttatcaacggtttatcaggatattaaagagaaactttctgccgaaattgtaatcaaacagaaggtagaactgtatcctaatatgtgtgtgacgaactttaccgaatctgaacaatgggatacggtaatagagggaaacgataaccttttagagaaatatatgtccggtaaatcattagaagcattggaactcgaacaagaggaaagcataagatttcagaattgttctctgttccctctttatcatggaagtgcaaaaagtaatatagggattgataaccttatagaagttattactaataaattttattcatcaacacatcgaggtccgtctgaactttgcggaaatgttttcaaaattgaatatacaaaaaaaagacaacgtcttgcatatatacgcctttatagtggagtactacatttacgagattcggttagagtatcagaaaaagaaaaaataaaagttacagaaatgtatacttcaataaatggtgaattatgtaagattgatagagcttattctggagaaattgttattttgcaaaatgagtttttgaagttaaatagtgttcttggagatacaaaactattgccacagagaaaaaagattgaaaatccgcaccctctactacaaacaactgttgaaccgagtaaacctgaacagagagaaatgttgcttgatgcccttttggaaatctcagatagtgatccgcttctacgatattacgtggattctacgacacatgaaattatactttctttcttagggaaagtacaaatggaagtgattagtgcactgttgcaagaaaagtatcatgtggagatagaactaaaagagcctacagtcatttatatggagagaccgttaaaaaatgcagaatataccattcacatcgaagtgccgccaaatcctttctgggcttccattggtttatctgtatcaccgcttccgttgggaagtggaatgcagtatgagagctcggtttctcttggatacttaaatcaatcatttcaaaatgcagttatggaaggggtacgctatggttgcgaacaaggattatatggttggaatgtgacggattgtaaaatctgttttaagtacggtttatactatagccctgttagtactccagcagattttcggatgcttactcctattgtactggagcaagcctttagaaaagctggaacagaattgttagagccatatcttagttttaaagtttatgcaccacaggaatatctttcncgggcatataacgatgctcccaaatattgtgcaaatatcgtaaatactcaactgaaaaataatgaggtcattattattggagaaattcctgctcgatgtattcaagattatcgcaatgatttaactttttttacaaatgggcttagtgtttgtttagcagagctaaaaggatatcaggttaccactggcgaacctgtttgccagacccgtcgtctaaatagtcggatagataaagtaagatatatgttcaataaaataacttagtgcgttttatgttgttatataaatatggtttcttattaaataagatgaaatattctttaatatagatttgaattaaagtggaaaggaggagattgttattataaactacaagtggatattgtgtcctatttgtggaaataaaacaagactacgaatacgagtggatactatacttaaaaatttccctttatacagccccaaatgtaagaacgaaactttaattaatgttcaaaaaatgaatataataacaatcaaagagccagacgccaagacgcagagccgataatttgagaaatgaaactctcatcttatcggctctttttgtttatctgaattttactgactagccttcaatatttcc

SEQ ID NO: 6 - DNA, 1194 bp, Enterobacteria phage P1
gtgacctgggacgatcacaagaagaattttgctcgcctggcgcgagatggtggttacaccatcgcacagtatgccgccgagtttaatcttaaccctaataccgcacgtcgttatctccgtgccttcaaagaagacaccaggactacggacagccgcaagccaaataagccagtcaggaagccactaaaaagcatgatcattgatcactctaatgatcaacatgcaggtgatcacattgcggctgaaatagcggaaaaacaaagagttaatgccgttgtcagtgccgcagtcgagaatgcgaagcgccaaaataagcgcataaatgatcgttcagatgatcatgacgtgatcacccgcgcccaccggaccttacgtgatcgcctggaacgcgacaccctggatgatgatggtgaacgctttgaattcgaagttggcgattacctgatagataacgttgaagcgcggaaggccgcgcgcgctatgttgcgtcggtccggggccgatgttctggaaaccactcttctggaaaagtctctttctcatctccttatgctggagaacgccagggatacgtgtattcgcctggtgcaggaaatgcgcgatcagcaaaaagacgatgatgaaggtactccgcctgaataccgtatcgcgagcatgctaaacagctgttccgcgcagataagcagcctgatcaacaccatttacagcatccggaataactatcgaaaagaaagccgggaggcggaaaagcacgctttatctatggggcaagctggcattgttaagctggcatacgaacgaaagcgtgaaaataactggtcagtgctggaagcggctgaattcatcgaggcgcatggaggaaaagtgccgcccctgatgctggagcaaatcaaagccgatctgcgtgctcctaagaccaataccgatgatgaggaaaaccaaacagcatctggcgctccatcacttgaagatctggataaaatcgcgcgagaacgggccgccagccgccgcgctgatgccgcattgtggattgagcatcgtagagaagaaattgccgatatcgtcgatacaggtggttatggtgatgtcgatgcggaaggcatatcaaacgaagcatggcttgaacaggatctggacgaagacgaggaggaagacgaagaagttacccgcaaactgtacggggatgatgattaa

SEQ ID NO: 7 - DNA, 1194 bp, Enterobacteria phage P1; identical to SEQ ID NO: 6

SEQ ID NO: 8 - DNA, 525 bp, Artificial Sequence
  Description of Artificial Sequence: Synthetic polynucleotide
atgaacgaaaaacaaaagagattcgcagatgaatatataatgaatggatgtaatggtaaaaaagcagcaatttcagcaggttatagtaagaaaacagcagagtctttagcaagtcgattgttaagaaatgttaatgtttcggaatatattaaagaacgattagaacagatacaagaagagcgtttaatgagcattacagaagctttagcgttatctgcttctattgctagaggagaacctcaagaggcttacagtaagaaatatgaccatttaaacgatgaagtggaaaaagaggttacttacacaatcacaccaacttttgaagagcgtcagagatctattgaccacatactaaaagttcatggtgcgtatatcgacaaaaaagaaattactcagaagaatattgagattaatattagatctattgaccacatactaaaagttcatggtgcgtatatcgacaaaaaagaaattactcagaagaatattgagattaatattggtgagtacgatgacgaaagttaa

SEQ ID NO: 9 - DNA, 663 bp, Staphylococcus phage 80alpha
aattggcagtaaagtggcagtttttgatacctaaaatgagatattatgatagtgtaggatattgactatcttactgcgtttcccttatcgcaattaggaataaaggatctatgtgggttggctgattatagccaatccttttttaattttaaaaagcgtatagcgcgagagttggtggtaaatgaaatgaacgaaaaacaaaagagattcgcagatgaatatataatgaatggatgtaatggtaaaaaagcagcaatttcagcaggttatagtaagaaaacagcagagtctttagcaagtcgattgttaagaaatgttaatgtttcggaatatattaaagaacgattagaacagatacaagaagagcgtttaatgagcattacagaagctttagcgttatctgcttctattgctagaggagaacctcaagaggcttacagtaagaaatatgaccatttaaacgatgaagtggaaaaagaggttacttacacaatcacaccaacttttgaagagcgtcagagatctattgaccacatactaaaagttcatggtgcgtatatcgacaaaaaagaaattactcagaagaatattgagattaatattggtgagtacgatgacgaaagttaaattaaactttaacaaaccatctaatgttttcaacag

SEQ ID NO: 10 - DNA, 1116 bp, Staphylococcus aureus
tcataaatatttaactatttctttctgtgtactagggtacaaatgaccgtatcggttatatacttcattactatcagcatggcctaaacgctgtgctattaccatgatacttgcgccatgattgactagcatagacgcatggctatgtcttaactcatgaattacaattctagggaatgtctgaccgtctggtagttgttcatctaatacttttaatgcagcggtaaaccaacgatctatagttgattcactataagctttgaagaatgtaccgaataatacataatcatctttatatacattgttttctttgtaccattttaaatattctttgatatcattcatcatgtgaacaggtaagtatatatcacgtattgctgcttttgttttaggggctgtcacttcaccgtgatagtctgttttgttaatatgtatgaaatcatcatcatagttaatatcacgccatgtgagggctctaatttcgcccttacgtgcaccagagtaaaacagtagcttaaagaataacttttgttgttgtgtagctaaagcctcatagaattgattgaattgttctaatgtccaatagttcaaacgcttatttgattctatttcaaagttacctactagagaggctacattttgctttagatcatgaaacttcatagcatggttaagtaacgatactaagaacacgtgcattttctttaggtactctccagagtgtccctcttttaacttcgtattctgaaacttcataatatcttgtgtagtcatattaaacacgtccatagacttaaaatagggtagcaaatggttgtttgtatgtgtctttaatgctttcacactagatgacttacgacgtgcagaataccactctatatactcatctacgagcttatcaaagggcagtttgtttatctgtcctacaccctctaactcgtccataatttcattacatttcttcaatgcctctttacgctgtttaaagccactcttttttatttctttacgttgattaaatttatcatagtattttatacgaaaatagtatgtaccacgtttagcgtctttatatatgttgtgggataggtttaagttgtgttctatgggaatcac

SEQ ID NO: 11 - DNA, 10844 bp, Artificial Sequence
  Description of Artificial Sequence: Synthetic polynucleotide
  modified_base (8807)..(8807): a, c, t, g, unknown or other
ctcgggccgtctcttgggcttgatcggccttcttgcgcatctcacgcgctcctgcggcggcctgtagggcaggctcatacccctgccgaaccgcttttgtcagccggtcggccacggcttccggcgtctcaacgcgctttgagattcccagcttttcggccaatccctgcggtgcataggcgcgtggctcgaccgcttgcgggctgatggtgacgtggcccactggtggccgctccagggcctcgtagaacgcctgaatgcgcgtgtgacgtgccttgctgccctcgatgccccgttgcagccctagatcggccacagcggccgcaaacgtggtctggtcgcgggtcatctgcgctttgttgccgatgaactccttggccgacagcctgccgtcctgcgtcagcggcaccacgaacgcggtcatgtgcgggctggtttcgtcacggtggatgctggccgtcacgatgcgatccgccccgtacttgtccgccagccacttgtgcgccttctcgaagaacgccgcctgctgttcttggctggccgacttccaccattccgggctggccgtcatgacgtactcgaccgccaacacagcgtccttgcgccgcttctctggcagcaactcgcgcagtcggcccatcgcttcatcggtgctgctggccgcccagtgctcgttctctggcgtcctgctggcgtcagcgttgggcgtctcgcgctcgcggtaggcgtgcttgagactggccgccacgttgcccattttcgccagcttcttgcatcgcatgatcgcgtatgccgccatgcctgcccctcccttttggtgtccaaccggctcgacgggggcagcgcaaggcggtgcctccggcgggccactcaatgcttgagtatactcactagactttgcttcgcaaagtcgtgaccgcctacggcggctgcggcgccctacgggcttgctctccgggcttcgccctgcgcggtcgctgcgctcccttgccagcccgtggatatgtggacgatggccgcgagcggccaccggctggctcgcttcgctcggcccgtggacaaccctgctggacaagctgatggacaggctgcgcctgcccacgagcttgaccacagggattgcccaccggctaccactatagggcgaattggcggaaggccgtcaaggccgcatttgggcccggcgcgccggatccgctagctctagacctctagaccagccaggacagaaatgcctcgacttcgctgctgcccaaggttgccgggtgacgcacaccgtggaaacggatgaaggcacgaacccagtggacataagcctgttcggttcgtaagctgtaatgcaagtagcgtgcccgttccgggccttttgacatgtgactttcgttaccctcgcgtcaaaaagagtttttacgaaaggaagcataagtgacctgggacgatcacaagaagaattttgctcgcctggcgcgagatggtggttacaccatcgcacagtatgccgccgagtttaatcttaaccctaataccgcacgtcgttatctccgtgccttcaaagaagacaccaggactacggacagccgcaagccaaataagccagtcaggaagccactaaaaagcatgatcattgatcactctaatgatcaacatgcaggtgatcacattgcggctgaaatagcggaaaaacaaagagttaatgccgttgtcagtgccgcagtcgagaatgcgaagcgccaaaataagcgcataaatgatcgttcagatgatcatgacgtgatcacccgcgcccaccggaccttacgtgatcgcctggaacgcgacaccctggatgatgatggtgaacgctttgaattcgaagttggcgattacctgatagataacgttgaagcgcggaaggccgcgcgcgctatgttgcgtcggtccggggccgatgttctggaaaccactcttctggaaaagtctctttctcatctccttatgctggagaacgccagggatacgtgtattcgcctggtgcaggaaatgcgcgatcagcaaaaagacgatgatgaaggtactccgcctgaataccgtatcgcgagcatgctaaacagctgttccgcgcagataagcagcctgatcaacaccatttacagcatccggaataactatcgaaaagaaagccgggaggcggaaaagcacgctttatctatggggcaagctggcattgttaagctggcatacgaacgaaagcgtgaaaataactggtcagtgctggaagcggctgaattcatcgaggcgcatggaggaaaagtgccgcccctgatgctggagcaaatcaaagccgatctgcgtgctcctaagaccaataccgatgatgaggaaaaccaaacagcatctggcgctccatcacttgaagatctggataaaatcgcgcgagaacgggccgccagccgccgcgctgatgccgcattgtggattgagcatcgtagagaagaaattgccgatatcgtcgatacaggtggttatggtgatgtcgatgcggaaggcatatcaaacgaagcatggcttgaacaggatctggacgaagacgaggaggaagacgaagaagttacccgcaaactgtacggggatgatgattaattaaaaaaacccgccccggcgggtttttttatctagagctagcggatccggcgcgccgggcccttctgggcctcatgggccttccgctcactgcccgctttccagcactatagggcgaattggcggaaggccgtcaaggccgcatttgggcccggcgcgccggatccgctagctctagactggcaggtttctgagcagatcgtccaacccgatctggatcgggtcagaaaaatttgctctaataaatttcgttttctaagtgcaaagaatcaccatttcgagctggtgattgaaggttgatgcaaatttggagaaaaaatgcaacaaacattcaatgcggatatgaatatatcaaaccttcatcaaaatgtcgatccttcaaccactctgcccgttatttgtggtgttgaaattacgaccgaccgcgctggccgttacaaccttaatgctctacacagagcgagcggactcggtgcccataaagcgccagctcaatggctaagaacgctgtcagctaaacagctcatcgaagagcttgaaaaagaaactatgcagaattgcatagtttcgttcacaagcaatggaagcaggatttctttcacgactcgtataaccggcaaaggtcagcagtggctgatgaagcgattgcttgatgctggtgtgctggtacctgtcgcggcaacgcgctaacagacgtagtaagaaccaccagcattgtaatgctggctaaagtcactttcctgagctgtataacgatgagcgattttactttttctggctatgaattggcctgctttgtaacacactccggtctatcccgtagcgccgggcatatcctgtcgcaatgtgcaaatctcgcggcaacaaccagtgaatacttcattcacaagcctcaccgcctgatcgcggcagaaactggttatagccaatcaaccgtcgttcgtgcattccgtgaagctgtaaacaaaggaattctgtctgtagagattgttatcggcgatcaccgtgaacgtcgcgctaacctgtaccggtttacaccatcctttttggccttcgcacaacaagccaaaaatgcgctgatagaaagcaaattaaagatctcttcagcggcaaccaaggttaaagctgttctcgctaagacattggctttatttaattttttatccacacccccatgtcaaaatgataccccctccccctgtcaggatgacgtggcaataaagaataagaagtcacaagttaaaaaaacaaaaagatcagtttccggcggtgccggaacaaccagcctcaaaaaattgacttcatggatcgctaaggcaaaagcaaaggctgacaatctgcggttatccaaaaaacgcactcaaaaacatgagttcaagcagaaagtagaggcggctgcgcggaaatatgcttacctgaagaacaagcgttcgcctgatattggcgggatatcaaacttcgataacctaccgcattgcatgacggtaaacgaagctcttaatgcggttttagccaaaaataaagataacgaacaatggggtataccggcaggattcagagggtaatgaattgctctaattataaccatgcatactttcaacacctctagtttgccatgaggcaaactcataggtgtcctggtaagaggacactgttgccaaaactggacgccccattattgcaattaataaacaactaacggacaattctacctaacaataagtggcttaaaaaaacccgccccggcgggtttttttatctagagctagcggatccggcgcgccgggcccttctgggcctcatgggccttccgctcactgcccgctttccagccagccttcgaccacatacccaccggctccaactgcgcggcctgcggccttgccccatcaatttttttaattttctctggggaaaagcctccggcctgcggcctgcgcgcttcgcttgccggttggacaccaagtggaaggcgggtcaaggctcgcgcagcgaccgcgcagcggcttggccttgacgcgcctggaacgacccaagcctatgcgagtgggggcagtcgaaggcgaagcccgcccgcctgccccccgagacctgcaggggggggggggcgctgaggtctgcctcgtgaagaaggtgttgctgactcataccaggcctgaatcgccccatcatccagccagaaagtgagggagccacggttgatgagagctttgttgtaggtggaccagttggtgattttgaacttttgctttgccacggaacggtctgcgttgtcgggaagatgcgtgatctgatccttcaactcagcaaaagttcgatttattcaacaaagccgccgtcccgtcaagtcagcgtaatgctctgccagtgttacaaccaattaaccaattctgattagaaaaactcatcgagcatcaaatgaaactgcaatttattcatatcaggattatcaataccatatttttgaaaaagccgtttctgtaatgaaggagaaaactcaccgaggcagttccataggatggcaagatcctggtatcggtctgcgattccgactcgtccaacatcaatacaacctattaatttcccctcgtcaaaaataaggttatcaagtgagaaatcaccatgagtgacgactgaatccggtgagaatggcaaaagcttatgcatttctttccagacttgttcaacaggccagccattacgctcgtcatcaaaatcactcgcatcaaccaaaccgttattcattcgtgattgcgcctgagcgagacgaaatacgcgatcgctgttaaaaggacaattacaaacaggaatcgaatgcaaccggcgcaggaacactgccagcgcatcaacaatattttcacctgaatcaggatattcttctaatacctggaatgctgttttcccggggatcgcagtggtgagtaaccatgcatcatcaggagtacggataaaatgcttgatggtcggaagaggcataaattccgtcagccagtttagtctgaccatctcatctgtaacatcattggcaacgctacctttgccatgtttcagaaacaactctggcgcatcgggcttcccatacaatcgatagattgtcgcacctgattgcccgacattatcgcgagcccatttatacccatataaatcagcatccatgttggaatttaatcgcggcctcgagcaagacgtttcccgttgaatatggctcataacaccccttgtattactgtttatgtaagcagacagttttattgttcatgatgatatatttttatcttgtgcaatgtaacatcagagattttgagacacaacgtggctttcccccccccccctgcaggtcccgagcctcacggcggcgagtgcgggggttccaagggggcagcgccaccttgggcaaggccgaaggccgcgcagtcgatcaacaagccccggaggggccactttttgccggagggggagccgcgccgaaggcgtgggggaaccccgcaggggtgcccttctttgggcaccaaagaactagatatagggcgaaatgcgaaagacttaaaaatcaacaacttaaaaaaggggggtacgcaacagctcattgcggcaccccccgcaatagctcattgcgtaggttaaagaaaatctgtaattgactgccacttttacgcaacgcataattgttgtcgcgctgccgaaaagttgcagctgattgcgcatggtgccgcaaccgtgcggcacccctaccgcatggagataagcatggccacgcagtccagagaaatcggcattcaagccaagaacaagcccggtcactgggtgcaaacggaacgcaaagcgcatgaggcgtgggccgggcttattgcgaggaaacccacggcggcaatgctgctgcatcacctcgtggcgcagatgggccaccagaacgccgtggtggtcagccagaagacactttccaagctcatcggacgttctttgcggacggtccaatacgcagtcaaggacttggtggccgagcgctggatctccgtcgtgaagctcaacggccccggcaccgtgtcggcctacgtggtcaatgaccgcgtggcgtggggccagccccgcgaccagttgcgcctgtcggtgttcagtgccgccgtggtggttgatcacgacgaccaggacgaatcgctgttggggcatggcgacctgcgccgcatcccgaccctgtatccgggcgagcagcaactaccgaccggccccggcgaggagccgcccagccagcccggcattccgggcatggaaccagacctgccagccttgaccgaaacggaggaatgggaacggcgcgggcagcagcgcctgccgatgcccgatgagccgtgttttctggacgatggcgagccgttggagccgccgacacgggtcacgctgccgcgccggtagcacttgggttgcgcagcaacccgtaagtgcgctgttccagactatcggctgtagccgcctcgccgccctataccttgtctgcctccccgcgttgcgtcgcggtgcatggagccgggccacctcgacctgaatggaagccggcggcacctcgctaacggattcaccgtttttatcaggctctgggaggcagaataaatgatcatatcgtcaattattacctccacggggagagcctgagcaaactggcctcaggcatttgagaagcacacggtcacactgcttccggtagtcaataaaccggtaaaccagcaatagacataagcggctatttaacgaccctgccctgaaccgacgaccgggtcgaatttgctttcgaatttctgccattcatccgcttattatacttattcaggcgtagcaccaggcgtttaagggcaccaataactgccttaaaaaaattacgccccgccctgccactcatcgcactcgtcaggtggcacttttcggggaaatgtgcgcggaacccctatttgtttatttttctaaatacattcaaatatgtatccgctcatgagacaataaccctgataaatgcttcaataatattgaaaaaggaagagtatgaagtttggaaatatttgtttttcgtatcaaccaccaggtgaaactcataagctaagtaatggatcgctttgttcggcttggtatcgcctcagaagagtagggtttgatacatattggaccttagaacatcattttacagagtttggtcttacgggaaatttatttgttgctgcggctaacctgttaggaagaactaaaacattaaatgttggcactatgggggttgttattccgacagcacacccagttcgacagttagaagacgttttattattagatcaaatgtcgaaaggtcgttttaattttggaaccgttcgagggctataccataaagattttcgagtatttggtgttgatatggaagagtctcgagcaattactcaaaatttctaccagatgataatggaaagcttacagacaggaaccattagctctgatagtgattacattcaatttcctaaggttgatgtatatcccaaagtgtactcaaaaaatgtaccaacctgtatgactgctgagtccgcaagtacgacagaatggctagcaatacaagggctaccaatggttcttagttggattattggtactaatgaaaaaaaagcacagatggaactctataatgaaattgcgacagaatatggtcatgatatatctaaaatagatcattgtatgacttatatttgttctgttgatgatgatgcacaaaaggcgcaagatgtttgtcgggagtttctgaaaaattggtatgactcatatgtaaatgcgaccaatatctttaatgatagcaatcaaactcgtggttatgattatcataaaggtcaatggcgtgattttgttttacaaggacatacaaacaccaatcgacgtgttgattatagcaatggtattaaccctgtaggcactcctgagcagtgtattgaaatcattcaacgtgatattgatgcaacgggtattacaaacattacatgcggatttgaagctaatggaactgaagatgaaataattgcttccatgcgacgctttatgacacaagtcgctcctttcttaaaagaacctaaataaattacttatttgatactagagataataaggaacaagttatgaaatttggattattttttctaaactttcagaaagatggaataacatctgangaaacgttggataatatggtaaagactgtcacgttaattgattcaactaaatatcattttaatactgcctttgttaatgaacatcacttttcaaaaaatggtattgttggagcacctattaccgcagctggttttttattagggttaacaaataaattacatattggttcattaaatcaagtaattaccacccatcaccctgtacgtgtagcagaagaagccagtttattagatcaaatgtcagagggacgcttcattcttggttttagtgactgcgaaagtgatttcgaaatggaattttttagacgtcatatctcatcaaggcaacaacaatttgaagcatgctatgaaataattaatgacgcattaactacaggttattgtcatccccaaaacgacttttatgattttccaaaggtttcaattaatccacactgttacagtgagaatggacctaagcaatatgtatccgctacatcaaaagaagtcgtcatgtgggcagcgaaaaaggcactgcctttaacatttaagtgggaggataatttagaaaccaaagaacgctatgcaattctatataataaaacagcacaacaatatggtattgatatttcggatgttgatcatcaattaactgtaattgcgaacttaaatgctgatagaagtacggctcaagaagaagtgagagaatacttaaaagactatatcactgaaacttaccctcaaatggacagagatgaaaaaattaactgcattattgaagagaatgcagttgggtctcatgatgactattatgaatcgacaaaattagcagtggaaaaaacagggtctaaaaatattttattatcctttgaatcaatgtccgatattaaagatgtaaaagatattattgatatgttgaaccaaaaaatcgaaatgaatttaccataaagtagtactgttgtaattcattaagcattctgccgacatggaagccatcacagacggcatgatgaacctgaatcgccagcggcatcagcaccttgtcgccttgcgtataatatttgcccatggtgaaaacgggggcgaagaagttgtccatattggccacgtttaaatcaaaactggtgaaactcacccagggattggctgagacgaaaaacatattctcaataaaccctttagggaaataggccaggttttcaccgtaacacgccacatcttgcgaatatatgtgtagaaactgccggaaatcgtcgtggtattcactccagagcgatgaaaacgtttcagtttgctcatggaaaacggtgtaacaagggtgaacactatcccatatcaccagctcaccgtctttcattgccatacggaattccggatgagcattcatcaggcgggcaagaatgtgaataaaggccggataaaacttgtgcttatttttctttacggtctttaaaaaggccgtaatatccagctgaacggtctggttataggtacattgagcaactgactgaaatgcctcaaaatgttctttacgatgccattgggatatatcaacggtggtatatccagtgatttttttctccattttagcttccttagctcctgaaaatctcgataactcaaaaaatacgcccggtagtgatcttatttcattatggtgaaagttggaacctcttacgtgccgatcaacgtctcattttcgccaaaagttggcccagggcttcccggtatcaacagggacaccaggatttatttattctgcgaagtgatcttccgtcacaggtatttattcgaagacgaaagggcctcgtgatacgcctatttttataggttaatgtcatgataataatggtttcttagacgtcaggtggcacttttcggggaaatgtgcgcgcccgcgttcctgctggcgctgggcctgtttctggcgctggacttcccgctgttccgtcagcagcttttcgcccacggccttgatgatcgcggcggccttggcctgcatatcccgattcaacggccccagggcgtccagaacgggcttcaggcgctcccgaaggt

SEQ ID NO: 12 - DNA, 128 bp, Staphylococcus aureus
gtctagttaatgtgtaacgtaacattagctagatttttttattcaaaaaaatatttacaaatattaggaaatttaagtgtaaaagagttgataaatgattatattgggactataatataattaaggtc

SEQ ID NO: 13 - DNA, 2769 bp, Staphylococcus phage 80alpha
attagacaacaaacaagtcattgaaaattccgacttattattcaaaaagaaatttgatagcgcagatatacaagctaggttaaaagtaggcgataaggtagaagttaaaacaatcggttatagaatacactttttaaatttatatccggtcttatacgaagtaaagaaggtagataaacaatgattaaacaaatactaagactattattcttactagcaatgtatgagttaggtaagtatgtaactgagcaagtatatattatgatgacggctaatgatgatgtagaggtgccgagtgacttcgcgaagttgagcgatcagtcagatttgatgagggcggaggtgacggagtagatgatgtggttagtcatagcaattatattactagtcatcttattgtttggtgtgatgttgcaagctgaacagttaaaaggcgatgtgaaagttaaagagcgggagatagagatattaagaagtagattgagacattttgaagattaaaaatatttgtatggagggtattcatgactaaaaagaaatatggattaaaattatcaacagttcgaaagttagaagatgagttgtgtgattatcctaattatcataagcaactcgaagatttaagaagtgaaataatgacaccatggattccaacagatacaaatataggcggggagtttgtaccgtctaatacatcgaaaacagaaatggcagtaactaattatctttgtagtatacgaagaggtaaaatccttgagtttaagagcgctattgaacgtataatcaacacatcaagtaggaaagaacgcgaattcattcaagagtattattttaataaaaaggaattagtgaaagtttgtgatgacatacacatttctgatagaactgctcatagaatcaaaaggaaaatcatatctagattggcggaagagttaggggaagagtgaaattggcagtaaagtggcagtttttgatacctaaaatgagatattatgatagtgtaggatattgactatcttactgcgtttcccttatcgcaattaggaataaaggatctatgtgggttggctgattatagccaatccttttttaattttaaaaagcgtatagcgcgagagttggtggtaaatgaaatgaacgaaaaacaaaagagattcgcagatgaatatataatgaatggatgtaatggtaaaaaagcagcaatttcagcaggttatagtaagaaaacagcagagtctttagcaagtcgattgttaagaaatgttaatgtttcggaatatattaaagaacgattagaacagatacaagaagagcgtttaatgagcattacagaagctttagcgttatctgcttctattgctagaggagaacctcaagaggcttacagtaagaaatatgaccatttaaacgatgaagtggaaaaagaggttacttacacaatcacaccaacttttgaagagcgtcagagatctattgaccacatactaaaagttcatggtgcgtatatcgacaaaaaagaaattactcagaagaatattgagattaatattggtgagtacgatgacgaaagttaaattaaactttaacaaaccatctaatgttttcaacagaaacatattcgaaatactaaccaattacgataacttcactgaagtacattacggtggaggttcgagtggtaagtctcacggcgttatacaaaaagttgtacttaaagcattgcaagactggaaatatcctaggcgtatactatggcttagaaaagtccaatcaacaattaaagatagtttattcgaagatgtcaaagattgtttgataaacttcggtatttgggacatgtgcctttggaataagactgataacaaagttgaattgccaaacggcgcagtttttttgtttaaaggattagataacccagagaaaataaagtcgataaaaggcatatcagacatagtcatggaagaagcgtctgaattcacactaaatgattacacgcaattaacgttgcgtttgagggagcgtaaacacgtgaataagcaaatatttttgatgtttaacccagtatctaaactgaattgggtttataagtatttctttgaacatggtgaaccaatggaaaatgtcatgattagacaatctagttatcgagataataagtttcttgatgaaatgacacgacaaaacttagagttgttagcaaatcgtaatccagcatattacaaaatttatgcgttaggtgaattttctacactagacaaattggttttccctaagtatgaaaaacgtttaataaataaagatgagttaagacatttaccttcttattttggattggactttggctacgttaatgatcctagtgcttttatacattctaaaatagatgtaaagaaaaagaagttatacatcattgaagagtatgttaaacaaggtatgctgaatgatgaaatagctaatgtcataaagcaacttggttatgctaaagaagaaattacagcagatagtgcagaacaaaaaagtatagctgaattaaggaatctagggcttaaaaggattttaccaaccaaaaaagggaagggctcggttgtacaagggttacaattcttaatgcaatttgaaatcattgttgatgaacgttgtttcaagactattgaagagtttgacaactacacatggcaaaaggacaaagatacaggtgaatataccaatgaaccagtagatacatacaatcattgtatcgattcgttgcgttattcagtggaacgattc

SEQ ID NO: 14 - DNA, 10319 bp, Artificial Sequence
  Description of Artificial Sequence: Synthetic polynucleotide
ggcgccatggttaagggccctttgcggaaagagttagtaagttaacagaagacgaaccaaaactaaatggtttagcaggaaacttagataaaaaaatgaatccagaattatattcagaacaggaacagcaacaagaacaacaaaagaatcaaaaacgagatagaggtatgcacttatagaacatgcatttatgccgagaaaacttattggttggaatgggctatgtgttagctaacttgttagcgagttggttggacttgaattgggattaatcccaagaaagtaccaactcaacaacacataaagccctgtaggttccgaccaataaggaaattggaataaagcaataaaaggagttgaagaaatgaaattcagagaagcctttgagaattttataacaagtaagtatgtacttggtgttttagtagtcttaactgtttaccagataatacaaatgcttaaataaaaaaagacttgatctgattagaccaaatcttttgatagtgttatattaataacaaaataaaaaggagtcgctcacgccctaccaaagtttgtgaacgacatcattcaaagaaaaaaacactgagttgtttttataatcttgtatatttagatattaaacgatatttaaatatacatcaagatatatatttgggtgagcgattacttaaacgaaattgagattaaggagtcgattttttatgtataaaaacaatcatgcaaatcattcaaatcatttggaaaatcacgatttagacaatttttctaaaaccggctactctaatagccggttggacgcacatactgtgtgcatatctgatccaaaattaagttttgatgcaatgacgatcgttggaaatctcaaccgagacaacgctcaggccctttctaaatttatgagtgtagagccccaaataagactttgggatattcttcaaacaaagtttaaagctaaagcacttcaagaaaaagtttatattgaatatgacaaagtgaaagcagatagttgggatagacgtaatatgcgtattgaatttaatccaaacaaacttacacgagatgaaatgatttggttaaaacaaaatataataagctacatggaagatgacggttttacaagattagatttagcctttgattttgaagatgatttgagtgactactatgcaatgtctgataaagcagttaagaaaactattttttatggtcgtaatggtaagccagaaacaaaatattttggcgtgagagatagtaatagatttattagaatttataataaaaagcaagaacgtaaagataatgcagatgctgaagttatgtctgaacatttatggcgtgtagaaatcgaacttaaaagagatatggtggattactggaatgattgctttagtgatttacatatcttgcaaccagattggaaaactatccaacgcactgcggatagagcaatagtttttatgttattgagtgatgaagaagaatggggaaagcttcacagaaattctagaacaaaatataagaatttgataaaagaaatttcgccagtcgatttaacggacttaatgaaatcgactttaaaagcgaacgaaaaacaattgcaaaaacaaatcgatttttggcaacatgaatttaaattttggaaatagtgtacatattaatattactgaacaaaaatgatatatttaaactattctaatttaggaggatttttttatgaagtgtctatttaaaaatttggggaatttatatgaggtgaaagaataatttacccctataaactttagccacctcaagtaaagaggtaaaattgtttagtttatataaaaaatttaaaggtttgttttatagcgttttattttggctttgtattctttcattttttagtgtattaaatgaaatggttttaaatgtttctttacctgatattgcaaatcattttaatactactcctggaattacaaactgggtaaacactgcatatatgttaactttttcgataggaacagcagtatatggaaaattatctgattatataaatataaaaaaattgttaattattggtattagtttgagctgtcttggttcattgattgcttttattgggcccacctaggcaaatatgctcttacgtgctattatttaagtgactatttaaaaggagttaataaatatgcggcaaggtattcttaaataaactgtcaatttgatagcgggaacaaataattagatgtccttttttaggagggcttagttttttgtacccagtttaagaatacctttatcatgtgattctaaagtatccagagaatatctgtatgctttgtatacctatggttatgcataaaaatcccagtgataaaagtatttatcactgggatttttatgcccttttgggtttttgaatggaggaaaatcacatgaaaattattaatattggagttttagctcatgttgatgcaggaaaaactaccttaacagaaagcttattatataacagtggagcgattacagaattaggaagcgtggacaaaggtacaacgaggacggataatacgcttttagaacgtcagagaggaattacaattcagacaggaataacctcttttcagtgggaaaatacgaaggtgaacatcatagacacgccaggacatatggatttcttagcagaagtatatcgttcattatcagttttagatggggcaattctactgatttctgcaaaagatggcgtacaagcacaaactcgtatattatttcatgcacttaggaaaatggggattcccacaatcttttttatcaataagattgaccaaaatggaattgatttatcaacggtttatcaggatattaaagagaaactttctgccgaaattgtaatcaaacagaaggtagaactgtatcctaatatgtgtgtgacgaactttaccgaatctgaacaatgggatacggtaatagagggaaacgataaccttttagagaaatatatgtccggtaaatcattagaagcattggaactcgaacaagaggaaagcataagatttcagaattgttctctgttccctctttatcatggaagtgcaaaaagtaatatagggattgataaccttatagaagttattactaataaattttattcatcaacacatcgaggtccgtctgaactttgcggaaatgttttcaaaattgaatatacaaaaaaaagacaacgtcttgcatatatacgcctttatagtggagtactacatttacgagattcggttagagtatcagaaaaagaaaaaataaaagttacagaaatgtatacttcaataaatggtgaattatgtaagattgatagagcttattctggagaaattgttattttgcaaaatgagtttttgaagttaaatagtgttcttggagatacaaaactattgccacagagaaaaaagattgaaaatccgcaccctctactacaaacaactgttgaaccgagtaaacctgaacagagagaaatgttgcttgatgcccttttggaaatctcagatagtgatccgcttctacgatattacgtggattctacgacacatgaaattatactttctttcttagggaaagtacaaatggaagtgattagtgcactgttgcaagaaaagtatcatgtggagatagaactaaaagagcctacagtcatttatatggagagaccgttaaaaaatgcagaatataccattcacatcgaagtgccgccaaatcctttctgggcttccattggtttatctgtatcgccgcttccgttgggaagtggaatgcagtatgagagctcggtttctcttggatacttaaatcaatcatttcaaaatgcagttatggaaggggtacgctatggttgcgaacaaggattatatggttggaatgtgacggattgtaaaatctgttttaagtacggtttatactatagccctgttagtactccagcagattttcggatgcttactcctattgtactggagcaagcctttagaaaagctggaacagaattgttagagccatatcttagttttaaagtttatgcaccacaggaatatctttcacgggcatataacgatgctcccaaatattgtgcaaatatcgtaaatactcaactgaaaaataatgaggtcattattattggagaaattcctgctcgatgtattcaagattatcgcaatgatttaactttttttacaaatgggcttagtgtttgtttagcagagctaaaaggatatcaggttaccactggcgaacctgtttgccagacccgtcgtctaaatagtcggatagataaagtaagatatatgttcaataaaataacttagtgcgttttatgttgttatataaatatggtttcttattaaataagatgaaatattctttaatatagatttgaattaaagtggaaaggaggagattgttattataaactacaagtggatattgtgtcctagttgtggaaataaaacaagactacgaatacgagtggatactatacttaaaaatttccctttatacagccccaaatgtaagaacgaaactttaattaatgttcaaaaaatgaatataataacaatcaaagagccagacgccaagacgcagagccgataatttgagaaatgaaactctcatcttatcggctctttttgtttatctgaattttactgactagccttcaatatttccgcggccagcttactatgccattattaagcttgtaatatcggagggtttattaattggcagtaaagtggcagtttttgataccttaaatgagatattatgatagtgtaggatattgactatcgtactgcgtttccctaccgcaaattaggaataaaggatctatgtgggttggctgattatagccaatccttttttaattttaaaaagcgtatagcgcgagagttggtggtaaatgaaatgaacgaaaaacaaaagagattcgcagatgaatatataatgaatggatgtaatggtaaaaaagcagcaattacagtaggttatagtaagaaaacagcagagtctttagcaagtcgattgttaagaaatgttaatgtttcggaatatattaaagaacgattagaacaggtacaagaagagcgtttaatgagtattacagaagctttagcgttatctgcttctattgctagaggagaacctcaagaggcttacagtaagaaatatgaccatttaaacgatgaagtggaaaaagaggttacttacacaatcacaccaacttttgaagagcgtcagagatctattgaccacatactaaaagtacatggtgcgtatatcgataaaaaagaaattactcagaagaatattgagattaatattggtgagtacgatgacgaaagttaaattgaactttaacaaaccgtctaatgttttcaatagccgcgggggcccaacacaccaacttttgaagagcgtcagagatctattgaccacatactaaaagtacatggtgcgtatatcgataaaaaagaaattactcagaagaatattgagattaatattggtgagtacgatgacgaaagttaaattaaactttaacaaaccgtctaatgttttcaatagccgcgggggcccaacgagcggccgcatagttaagccagccccgacacccgccaacacccgctgacgcgccctgacgggcttgtctgctcccggcatccgcttacagacaagctgtgaccgtctccgggagctgcatgtgtcagaggttttcaccgtcatcaccgaaacgcgcgagacgaaagggcctcgtgatacgcctatttttataggttaatgtcatgataataatggtttcttagacgtcaggtggcacttttcggggaaatgtgcgcggaacccctatttgtttatttttctaaatacattcaaatatgtatccgctcatgagacaataaccctgataaatgcttcaataatattgaaaaaggaagagtatgagtattcaacatttccgtgtcgcccttattcccttttttgcggcattttgccttcctgtttttgctcacccagaaacgctggtgaaagtaaaagatgctgaagatcagttgggtgcacgagtgggttacatcgaactggatctcaacagcggtaagatccttgagagttttcgccccgaagaacgttttccaatgatgagcacttttaaagttctgctatgtggcgcggtattatcccgtattgacgccgggcaagagcaactcggtcgccgcatacactattctcagaatgacttggttgagtactcaccggtcacagaaaagcatcttacggatggcatgacagtaagagaattatgcagtgctgccataaccatgagtgataacactgcggccaacttacttctgacaacgatcggaggaccgaaggagctaaccgcttttttgcacaacatgggggatcatgtaactcgccttgatcgttgggaaccggagctgaatgaagccataccaaacgacgagcgtgacaccacgatgcctgtagcaatggcaacaacgttgcgcaaactattaactggcgaactacttactctagcttcccggcaacaattaatagactggatggaggcggataaagttgcaggaccacttctgcgctcggcccttccggctggctggtttattgctgataaatctggagccggtgagcgtgggtctcgcggtatcattgcagcactggggccagatggtaagccctcccgtatcgtagttatctacacgacggggagtcaggcaactatggatgaacgaaatagacagatcgctgagataggtgcctcactgattaagcattggtaactgtcagaccaagtttactcatatatactttagattgatttaaaacttcatttttaatttaaaaggatctaggtgaagatcctttttgataatctcatgaccaaaatcccttaacgtgagttttcgttccactgagcgtcagaccccgtagaaaagatcaaaggatcttcttgagatcctttttttctgcgcgtaatctgctgcttgcaaacaaaaaaaccaccgctaccagcggtggtttttttgccggatcaagagctaccaactctttttccgaaggtaactggcttcagcagagcgcagataccaaatactgttcttctagtgtagccgtagttaggccaccacttcaagaactctgtagcaccgcctacatacctcgctctgctaatcctgttaccagtggctgctgccagtggcgataagtcgtgtcttaccgggttggactcaagacgatagttaccggataaggcgcagcggtcgggctgaacggggggttcgtgcacacagcccagcttggagcgaacgacctacaccgaacctgagatacctacagcgtgagctatgagaaagcgccacgcttcccgaagggagaaaggcggacaggtatccggtaagcggcagggtcggaacaggagagcgcacgagggagcttccagggggaaacgcctggtatctttatagtcctgtcgggtttcgccacctctgacttgagcgtcgatttttgtgatgctcgtcaggggggcggagcctatggaaaaacgccagcaacgcggcctttttacggttcctggccttttgctggccttttgctcacatgttctttcctgcgttatcccctgattctgtggataaccgtattaccgcctttgagtgagctggcgggtctagttaatgtgtaacgtaacattagctagatttttttattcaaaaaaatatttacaaatattaggaaatttaagtgtaaaagagttgataaatgattatattgggactataatataattaaggtcgattgaattcgttaactaattaatcaccaaaaaggaatagagtatgaagtttggaaatatttgtttttcgtatcaaccaccaggtgaaactcataagcaagtaatggatcgctttgttcggcttggtatcgcctcagaagaggtagggtttgatacatattggaccttagaacatcattttacagagtttggtcttacgggaaatttatttgttgctgcggctaacctgttaggaagaactaaaacattaaatgttggcactatgggggttgttattccgacagcacacccagttcgacagttagaagacgttttattattagatcaaatgtcgaaaggtcgttttaattttggaaccgttcgagggctataccataaagattttcgagtatttggtgttgatatggaagagtctcgagcaattactcaaaatttctaccagatgataatggaaagcttacagacaggaaccattagctctgatagtgattacattcaatttcctaaggttgatgtatatcccaaagtgtactcaaaaaatgtaccaacctgtatgactgctgagtccgcaagtacgacagaatggctagcaatacaagggctaccaatggttcttagttggattattggtactaatgaaaaaaaagcacagatggaactctataatgaaattgcgacagaatatggtcatgatatatctaaaatagatcattgtatgacttatatttgttctgttgatgatgatgcacaaaaggcgcaagatgtttgtcgggagtttctgaaaaattggtatgactcatatgtaaatgcgaccaatatctttaatgatagcaatcaaactcgtggttatgattatcataaaggtcaatggcgtgattttgttttacaaggacatacaaacaccaatcgacgtgttgattatagcaatggtattaaccccgtaggcactcctgagcagtgtattgaaatcattcaacgtgatattgatgcaacgggtattacaaacattacatgcggatttgaagctaatggaactgaagatgaaataattgcttccatgcgacgctttatgacacaagtcgctcctttcttaaaagaacctaaataaattacttatttgatactagagataataaggaacaagttatgaaatttggattattttttctaaactttcagaaagatggaataacatctgaagaaacgttggataatatggtaaagactgtcacgttaattgattcaactaaatatcattttaatactgcctttgttaatgaacatcacttttcaaaaaatggtattgttggagcacctattaccgcagctggttttttattagggttaacaaataaattacatattggttcattaaatcaagtaattaccacccatcaccctgtacgtgtagcagaagaagccagtttattagatcaaatgtcagagggacgcttcattcttggttttagtgactgcgaaagtgatttcgaaatggaattttttagacgtcatatctcatcaaggcaacaacaatttgaagcatgctatgaaataattaatgacgcattaactacaggttattgccatccccaaaacgacttttatgattttccaaaggtttcaattaatccacactgttacagtgagaatggacctaagcaatatgtatccgctacatcaaaagaagtcgtcatgtgggcagcgaaaaaggcactgcctttaacgtttaagtgggaggataatttagaaaccaaagaacgctatgcaattctatataataaaacagcacaacaatatggtattgatatttcggatgttgatcatcaattaactgtaattgcgaacttaaatgctgatagaagtacggctcaagaagaagtgagagaatacttaaaagactatatcactgaaacttaccctcaaatggacagagatgaaaaaattaactgcattattgaagagaatgcagttgggtctcatgatgactattatgaatcgacaaaattagcagtggaaaaaacagggtctaaaaatattttattatcctttgaatcaatgtccgatattaaagatgtaaaagatattattgatatgttgaaccaaaaaatcgaaatgaatttaccataataaaattaaaggcaatttctatattagattgcctttttggcgcgcctattctaatgcataataaatactgataacatcttatattttgtattatattttgtattatcgttgacatgtataattttgatatcaaaaactgattttccctctattattttcgagatttattttcttaattctctttaacaaactagaaatattgtatatacaaaaaattataaataatagatgaatagtttaattataggtgttcatcaatcgaaaaagcaacgtatcttatttaaagtgcgttgcttttttctcatttataaggttaaataattctcatatatcaagcaaagtgaca

SEQ ID NO: 15 - DNA, 2088 bp, Staphylococcus aureus
tatactacaaatgtagtcttatataaggaggatattgatgaaaaagataaaaattgttccacttattttaatagttgtagttgtcgggtttggtatatatttttatgcttcaaaagataaagaaattaataatactattgatgcaattgaagataaaaatttcaaacaagtttataaagatagcagttatatttctaaaagcgataatggtgaagtagaaatgactgaacgtccgataaaaatatataatagtttaggcgttaaagatataaacattcaggatcgtaaaataaaaaaagtatctaaaaataaaaaacgagtagatgctcaatataaaattaaaacaaactacggtaacattgatcgcaacgttcaatttaattttgttaaagaagatggtatgtggaagttagattgggatcatagcgtcattattccaggaatgcagaaagaccaaagcatacatattgaaaatttaaaatcagaacgtggtaaaattttagaccgaaacaatgtggaattggccaatacaggaacagcatatgagataggcatcgttccaaagaatgtatctaaaaaagattataaagcaatcgctaaagaactaagtatttctgaagactatatcaaacaacaaatggatcaaaattgggtacaagatgataccttcgttccacttaaaaccgttaaaaaaatggatgaatatttaagtgatttcgcaaaaaaatttcatcttacaactaatgaaacagaaagtcgtaactatcctctagaaaaagcgacttcacatctattaggttatgttggtcccattaactctgaagaattaaaacaaaaagaatataaaggctataaagatgatgcagttattggtaaaaagggactcgaaaaactttacgataaaaagctccaacatgaagatggctatcgtgtcacaatcgttgacgataatagcaatacaatcgcacatacattaatagagaaaaagaaaaaagatggcaaagatattcaactaactattgatgctaaagttcaaaagagtatttataacaacatgaaaaatgattatggctcaggtactgctatccaccctcaaacaggtgaattattagcacttgtaagcacaccttcatatgacgtctatccatttatgtatggcatgagtaacgaagaatataataaattaaccgaagataaaaaagaacctctgctcaacaagttccagattacaacttcaccaggttcaactcaaaaaatattaacagcaatgattgggttaaataacaaaacattagacgataaaacaagttataaaatcgatggtaaaggttggcaaaaagataaatcttggggtggttacaacgttacaagatatgaagtggtaaatggtaatatcgacttaaaacaagcaatagaatcatcagataacattttctttgctagagtagcactcgaattaggcagtaagaaatttgaaaaaggcatgaaaaaactaggtgttggtgaagatataccaagtgattatccattttataatgctcaaatttcaaacaaaaatttagataatgaaatattattagctgattcaggttacggacaaggtgaaatactgattaacccagtacagatcctttcaatctatagcgcattagaaaataatggcaatattaacgcacctcacttattaaaagacacgaaaaacaaagtttggaagaaaaatattatttccaaagaaaatatcaatctattaactgatggtatgcaacaagtcgtaaataaaacacataaagaagatatttatagatcttatgcaaacttaattggcaaatccggtactgcagaactcaaaatgaaacaaggagaaactggcagacaaattgggtggtttatatcatatgataaagataatccaaacatgatgatggctattaatgttaaagatgtacaagataaaggaatggctagctacaatgccaaaatctcaggtaaagtgtatgatgagctatatgagaacggtaataaaaaatacgatatagatgaataacaaaacagtgaagcaatccgtaacgatggttgcttcactgtttt

SEQ ID NO: 16 - RNA, 2075 nt, Staphylococcus aureus
uagucuuauauaaggaggauauugaugaaaaagauaaaaauuguuccacuuauuuuaauaguuguaguugucggguuugguauauauuuuuaugcuucaaaagauaaagaaauuaauaauacuauugaugcaauugaagauaaaaauuucaaacaaguuuauaaagauagcaguuauauuucuaaaagcgauaauggugaaguagaaaugacugaacguccgauaaaaauauauaauaguuuaggcguuaaagauauaaacauucaggaucguaaaauaaaaaaaguaucuaaaaauaaaaaacgaguagaugcucaauauaaaauuaaaacaaacuacgguaacauugaucgcaacguucaauuuaauuuuguuaaagaagaugguauguggaaguuagauugggaucauagcgucauuauuccaggaaugcagaaagaccaaagcauacauauugaaaauuuaaaaucagaacgugguaaaauuuuagaccgaaacaauguggaauuggccaauacaggaacagcauaugagauaggcaucguuccaaagaauguaucuaaaaaagauuauaaagcaaucgcuaaagaacuaaguauuucugaagacuauaucaaacaacaaauggaucaaaauuggguacaagaugauaccuucguuccacuuaaaaccguuaaaaaaauggaugaauauuuaagugauuucgcaaaaaaauuucaucuuacaacuaaugaaacagaaagucguaacuauccucuagaaaaagcgacuucacaucuauuagguuauguuggucccauuaacucugaagaauuaaaacaaaaagaauauaaaggcuauaaagaugaugcaguuauugguaaaaagggacucgaaaaacuuuacgauaaaaagcuccaacaugaagauggcuaucgugucacaaucguugacgauaauagcaauacaaucgcacauacauuaauagagaaaaagaaaaaagauggcaaagauauucaacuaacuauugaugcuaaaguucaaaagaguauuuauaacaacaugaaaaaugauuauggcucagguacugcuauccacccucaaacaggugaauuauuagcacuuguaagcacaccuucauaugacgucuauccauuuauguauggcaugaguaacgaagaauauaauaaauuaaccgaagauaaaaaagaaccucugcucaacaaguuccagauuacaacuucaccagguucaacucaaaaaauauuaacagcaaugauuggguuaaauaacaaaacauuagacgauaaaacaaguuauaaaaucgaugguaaagguuggcaaaaagauaaaucuuggggugguuacaacguuacaagauaugaagugguaaaugguaauaucgacuuaaaacaagcaauagaaucaucagauaacauuuucuuugcuagaguagcacucgaauuaggcaguaagaaauuugaaaaaggcaugaaaaaacuagguguuggugaagauauaccaagugauuauccauuuuauaaugcucaaauuucaaacaaaaauuuagauaaugaaauauuauuagcugauucagguuacggacaaggugaaauacugauuaacccaguacagauccuuucaaucuauagcgcauuagaaaauaauggcaauauuaacgcaccucacuuauuaaaagacacgaaaaacaaaguuuggaagaaaaauauuauuuccaaagaaaauaucaaucuauuaacugaugguaugcaacaagucguaaauaaaacacauaaagaagauauuuauagaucuuaugcaaacuuaauuggcaaauccgguacugcagaacucaaaaugaaacaaggagaaacuggcagacaaauugggugguuuauaucauaugauaaagauaauccaaacaugaugauggcuauuaauguuaaagauguacaagauaaaggaauggcuagcuacaaugccaaaaucucagguaaaguguaugaugagcuauaugagaacgguaauaaaaaauacgauauagaugaauaacaaaacagugaagcaauccguaacgaugguugcuucacuguuuu

SEQ ID NO: 17 - DNA, 2166 bp, Vibrio fischeri
  modified_base (1194)..(1194): a, c, t, g, unknown or other
ggcttaaataaacagaatcaccaaaaaggaatagagtatgaagtttggaaatatttgtttttcgtatcaaccaccaggtgaaactcataagctaagtaatggatcgctttgttcggcttggtatcgcctcagaagagtagggtttgatacatattggaccttagaacatcattttacagagtttggtcttacgggaaatttatttgttgctgcggctaacctgttaggaagaactaaaacattaaatgttggcactatgggggttgttattccgacagcacacccagttcgacagttagaagacgttttattattagatcaaatgtcgaaaggtcgttttaattttggaaccgttcgagggctataccataaagattttcgagtatttggtgttgatatggaagagtctcgagcaattactcaaaatttctaccagatgataatggaaagcttacagacaggaaccattagctctgatagtgattacattcaatttcctaaggttgatgtatatcccaaagtgtactcaaaaaatgtaccaacctgtatgactgctgagtccgcaagtacgacagaatggctagcaatacaagggctaccaatggttcttagttggattattggtactaatgaaaaaaaagcacagatggaactctataatgaaattgcgacagaatatggtcatgatatatctaaaatagatcattgtatgacttatatttgttctgttgatgatgatgcacaaaaggcgcaagatgtttgtcgggagtttctgaaaaattggtatgactcatatgtaaatgcgaccaatatctttaatgatagcaatcaaactcgtggttatgattatcataaaggtcaatggcgtgattttgttttacaaggacatacaaacaccaatcgacgtgttgattatagcaatggtattaaccctgtaggcactcctgagcagtgtattgaaatcattcaacgtgatattgatgcaacgggtattacaaacattacatgcggatttgaagctaatggaactgaagatgaaataattgcttccatgcgacgctttatgacacaagtcgctcctttcttaaaagaacctaaataaattacttatttgatactagagataataaggaacaagttatgaaatttggattattttttctaaactttcagaaagatggaataacatctgangaaacgttggataatatggtaaagactgtcacgttaattgattcaactaaatatcattttaatactgcctttgttaatgaacatcacttttcaaaaaatggtattgttggagcacctattaccgcagctggttttttattagggttaacaaataaattacatattggttcattaaatcaagtaattaccacccatcaccctgtacgtgtagcagaagaagccagtttattagatcaaatgtcagagggacgcttcattcttggttttagtgactgcgaaagtgatttcgaaatggaattttttagacgtcatatctcatcaaggcaacaacaatttgaagcatgctatgaaataattaatgacgcattaactacaggttattgtcatccccaaaacgacttttatgattttccaaaggtttcaattaatccacactgttacagtgagaatggacctaagcaatatgtatccgctacatcaaaagaagtcgtcatgtgggcagcgaaaaaggcactgcctttaacatttaagtgggaggataatttagaaaccaaagaacgctatgcaattctatataataaaacagcacaacaatatggtattgatatttcggatgttgatcatcaattaactgtaattgcgaacttaaatgctgatagaagtacggctcaagaagaagtgagagaatacttaaaagactatatcactgaaacttaccctcaaatggacagagatgaaaaaattaactgcattattgaagagaatgcagttgggtctcatgatgactattatgaatcgacaaaattagcagtggaaaaaacagggtctaaaaatattttattatcctttgaatcaatgtccgatattaaagatgtaaaagatattattgatatgttgaaccaaaaaatcgaaatgaatttaccataataaaattaaaggcaatttctatattagattgcctttttaaatttc

SEQ ID NO: 18 - RNA, 2143 nt, Vibrio fischeri
aaucaccaaaaaggaauagaguaugaaguuuggaaauauuuguuuuucguaucaaccaccaggugaaacucauaagcuaaguaauggaucgcuuuguucggcuugguaucgccucagaagaguaggguuugauacauauuggaccuuagaacaucauuuuacagaguuuggucuuacgggaaauuuauuuguugcugcggcuaaccuguuaggaagaacuaaaacauuaaauguuggcacuauggggguuguuauuccgacagcacacccaguucgacaguuagaagacguuuuauuauuagaucaaaugucgaaaggucguuuuaauuuuggaaccguucgagggcuauaccauaaagauuuucgaguauuugguguugauauggaagagucucgagcaauuacucaaaauuucuaccagaugauaauggaaagcuuacagacaggaaccauuagcucugauagugauuacauucaauuuccuaagguugauguauaucccaaaguguacucaaaaaauguaccaaccuguaugacugcugaguccgcaaguacgacagaauggcuagcaauacaagggcuaccaaugguucuuaguuggauuauugguacuaaugaaaaaaaagcacagauggaacucuauaaugaaauugcgacagaauauggucaugauauaucuaaaauagaucauuguaugacuuauauuuguucuguugaugaugaugcacaaaaggcgcaagauguuugucgggaguuucugaaaaauugguaugacucauauguaaaugcgaccaauaucuuuaaugauagcaaucaaacucgugguuaugauuaucauaaaggucaauggcgugauuuuguuuuacaaggacauacaaacaccaaucgacguguugauuauagcaaugguauuaacccuguaggcacuccugagcaguguauugaaaucauucaacgugauauugaugcaacggguauuacaaacauuacaugcggauuugaagcuaauggaacugaagaugaaauaauugcuuccaugcgacgcuuuaugacacaagucgcuccuuucuuaaaagaaccuaaauaaauuacuuauuugauacuagagauaauaaggaacaaguuaugaaauuuggauuauuuuuucuaaacuuucagaaagauggaauaacaucugaagaaacguuggauaauaugguaaagacugucacguuaauugauucaacuaaauaucauuuuaauacugccuuuguuaaugaacaucacuuuucaaaaaaugguauuguuggagcaccuauuaccgcagcugguuuuuuauuaggguuaacaaauaaauuacauauugguucauuaaaucaaguaauuaccacccaucacccuguacguguagcagaagaagccaguuuauuagaucaaaugucagagggacgcuucauucuugguuuuagugacugcgaaagugauuucgaaauggaauuuuuuagacgucauaucucaucaaggcaacaacaauuugaagcaugcuaugaaauaauuaaugacgcauuaacuacagguuauugucauccccaaaacgacuuuuaugauuuuccaaagguuucaauuaauccacacuguuacagugagaauggaccuaagcaauauguauccgcuacaucaaaagaagucgucaugugggcagcgaaaaaggcacugccuuuaacauuuaagugggaggauaauuuagaaaccaaagaacgcuaugcaauucuauauaauaaaacagcacaacaauaugguauugauauuucggauguugaucaucaauuaacuguaauugcgaacuuaaaugcugauagaaguacggcucaagaagaagugagagaauacuuaaaagacuauaucacugaaacuuacccucaaauggacagagaugaaaaaauuaacugcauuauugaagagaaugcaguugggucucaugaugacuauuaugaaucgacaaaauuagcaguggaaaaaacagggucuaaaaauauuuuauuauccuuugaaucaauguccgauauuaaagauguaaaagauauuauugauauguugaaccaaaaaaucgaaaugaauuuaccauaauaaaauuaaaggcaauuucuauauuagauugccuuuu

SEQ ID NO: 19 - RNA, 2294 nt, Artificial Sequence
  Description of Artificial Sequence: Synthetic polynucleotide
aaaggcaugaaaaaacuugguaucuucaccaacaccuagcuuuuugaaggaauugaguaugaaguuuggaaauauugguuguucguaucaaccaccaggugaaacucauaagcuaaaggcaugaaaaaacuaggugaucuucaccaacaccuaguuuuuucaaggaauugaguaugaaguuuggaaauauuuguuuuucguaucaaccaccaggugaaacucauaagcuaaguaauggaucgcuuuguucggcuugguaucgccucagaagaguaggguuugauacauauuggaccuuagaacaucauuuuacagaguuuggucuuacgggaaauuuauuuguugcugcggcuaaccuguuaggaagaacuaaaacauuaaauguuggcacuauggggguuguuauuccgacagcacacccaguucgacaguuagaagacguuuuauuauuagaucaaaugucgaaaggucguuuuaauuuuggaaccguucgagggcuauaccauaaagauuuucgaguauuugguguugauauggaagagucucgagcaauuacucaaaauuucuaccagaugauaauggaaagcuuacagacaggaaccauuagcucugauagugauuacauucaauuuccuaagguugauguauaucccaaaguguacucaaaaaauguaccaaccuguaugacugcugaguccgcaaguacgacagaauggcuagcaauacaagggcuaccaaugguucuuaguuggauuauugguacuaaugaaaaaaaagcacagauggaacucuauaaugaaauugcgacagaauauggucaugauauaucuaaaauagaucauuguaugacuuauauuuguucuguugaugaugaugcacaaaaggcgcaagauguuugucgggaguuucugaaaaauugguaugacucauauguaaaugcgaccaauaucuuuaaugauagcaaucaaacucgugguuaugauuaucauaaaggucaauggcgugauuuuguuuuacaaggacauacaaacaccaaucgacguguugauuauagcaaugguauuaacccuguaggcacuccugagcaguguauugaaaucauucaacgugauauugaugcaacggguauuacaaacauuacaugcggauuugaagcuaauggaacugaagaugaaauaauugcuuccaugcgacgcuuuaugacacaagucgcuccuuucuuaaaagaaccuaaauaaauuacuuauuugauacuagagauaauaaggaacaaguuaugaaauuuggauuauuuuuucuaaacuuucagaaagauggaauaacaucugaagaaacguuggauaauaugguaaagacugucacguuaauugauucaacuaaauaucauuuuaauacugccuuuguuaaugaacaucacuuuucaaaaaaugguauuguuggagcaccuauuaccgcagcugguuuuuuauuaggguuaacaaauaaauuacauauugguucauuaaaucaaguaauuaccacccaucacccuguacguguagcagaagaagccaguuuauuagaucaaaugucagagggacgcuucauucuugguuuuagugacugcgaaagugauuucgaaauggaauuuuuuagacgucauaucucaucaaggcaacaacaauuugaagcaugcuaugaaauaauuaaugacgcauuaacuacagguuauugucauccccaaaacgacuuuuaugauuuuccaaagguuucaauuaauccacacuguuacagugagaauggaccuaagcaauauguauccgcuacaucaaaagaagucgucaugugggcagcgaaaaaggcacugccuuuaacauuuaagugggaggauaauuuagaaaccaaagaacgcuaugcaauucuauauaauaaaacagcacaacaauaugguauugauauuucggauguugaucaucaauuaacuguaauugcgaacuuaaaugcugauagaaguacggcucaagaagaagugagagaauacuuaaaagacuauaucacugaaacuuacccucaaauggacagagaugaaaaaauuaacugcauuauugaagagaaugcaguugggucucaugaugacuauuaugaaucgacaaaauuagcaguggaaaaaacagggucuaaaaauauuuuauuauccuuugaaucaauguccgauauuaaagauguaaaagauauuauugauauguugaaccaaaaaaucgaaaugaauuuaccauaauaaaauuaaaggcaauuucuauauuagauugccuuuu

SEQ ID NO: 20 - RNA, 12 nt, Artificial Sequence
  Description of Artificial Sequence: Synthetic oligonucleotide
  modified_base (1)..(2): a, c, u, g, unknown or other
  modified_base (7)..(9): a, c, u, g, unknown or other
  modified_base (12)..(12): a, c, u, g, unknown or other
  See specification as filed for detailed description of substitutions and preferred embodiments
nnwawgnnnuun

SEQ ID NO: 21 - RNA, 13 nt, Artificial Sequence
  Description of Artificial Sequence: Synthetic oligonucleotide
  modified_base (1)..(1): a, c, u, g, unknown or other
  modified_base (4)..(7): a, c, u, g, unknown or other
  modified_base (12)..(13): a, c, u, g, unknown or other
  See specification as filed for detailed description of substitutions and preferred embodiments
nagnnnncwuwnn

SEQ ID NO: 22 - RNA, 13 nt, Artificial Sequence
  Description of Artificial Sequence: Synthetic oligonucleotide
cagauaacauuuu